European Patent Application EP 4 796 119 A1, published August 26, 2026. Title: TREATMENT OF OBESITY. Applicant: CYN-K BIO, INC. The sequence listing filed with the application follows.

SEQUENCE LISTING (16 sequences)

SEQ ID NO: 1 - protein, 250 aa, Homo sapiens [sequence omitted]

SEQ ID NO: 2 - protein, 30 aa, Homo sapiens
ADNFSLHDALSGSGNPNPQGWPGAWGNQPA

SEQ ID NO: 3 - protein, 34 aa, Homo sapiens
YPGASYPGAYPGQAPPGAYPGQAPPGAYPGAPGA

SEQ ID NO: 4 - protein, 74 aa, Homo sapiens
YPGASYPGAYPGQAPPGAYPGQAPPGAYPGAPGAYPGAPAPGVYPGPPSGPGAYPSSGQPSATGAYPATGPYGA

SEQ ID NO: 5 - protein, 30 aa, Mus musculus
ADSFSLNDALAGSGNPNPQGYPGAWGNQPA

SEQ ID NO: 6 - protein, 1248 aa, Chikungunya virus
MEFIPTQTFYNRRYQPRPWTPRPTIQVIRPRPRPQRQAGQLAQLISAVNKLTMRAVPQQKPRRNRKNKKQKQKQQAPQNNTNQKKQPPKKKPAQKKKKPGRRERMCMKIENDCIFEVKHEGKVTGYACLVGDKVMKPAHVKGTIDNADLAKLAFKRSSKYDLECAQIPVHMKSDASKFTHEKPEGYYNWHHGAVQYSGGRFTIPTGAGKPGDSGRPIFDNKGRVVAIVLGGANEGARTALSVVTWNKDIVTKITPEGAEEWSLAIPVMCLLANTTFPCSQPPCTPCCYEKEPEETLRMLEDNVMRPGYYQLLQASLTCSPHRQRRSTKDNFNVYKATRPYLAHCPDCGEGHSCHSPVALERIRNEATDGTLKIQVSLQIGIKTDDSHDWTKLRYMDNHMPADAERAGLFVRTSAPCTITGTMGHFILARCPKGETLTVGFTDSRKISHSCTHPFHHDPPVIGREKFHSRPQHGKELPCSTYVQSTAATTEEIEVHMPPDTPDRTLMSQQSGNVKITVNGQTVRYKCNCGGSNEGLTTTDKVINNCKVDQCHAAVTNHKKWQYNSPLVPRNAELGDRKGKIHIPFPLANVTCRVPKARNPTVTYGKNQVIMLLYPDHPTLLSYRNMGEEPNYQEEWVMHKKEVVLTVPTEGLEVTWGNNEPYKYWPQLSTNGTAHGHPHEIILYYYELYPTMTVVVVSVATFILLSMVGMAAGMCMCARRRCITPYELTPGATVPFLLSLICCIRTAKAATYQEAAIYLWNEQQPLFWLQALIPLAALIVLCNCLRLLPCCCKTLAFLAVMSVGAHTVSAYEHVTVIPNTVGVPYKTLVNRPGYSPMVLEMELLSVTLEPTLSLDYITCEYKTVIPSPYVKCCGTAECKDKNLPDYSCKVFTGVYPFMWGGAYCFCDAENTQLSEAHVEKSESCKTEFASAYRAHTASASAKLRVLYQGNNITVTAYANGDHAVTVKDAKFIVGPMSSAWTPFDNKIVVYKGDVYNMDYPPFGAGRPGQFGDIQSRTPESKDVYANTQLVLQRPAVGTVHVPYSQAPSGFKYWLKERGASLQHTAPFGCQIATNPVRAVNCAVGNMPISIDIPEAAFTRVVDAPSLTDMSCEVPACTHSSDFGGVAIIKYAASKKGKCAVHSMTNAVTIREAEIEVEGNSQLQISFSTALASAEFRVQVCSTQVHCAAECHPPKDHIVNYPASHTTLGVQDISATAMSWVQKITGGVGLVVAVAALILIVVLCVSFSRH

SEQ ID NO: 7 - protein, 1248 aa, Chikungunya virus
MEFIPTQTFYNRRYQPRPWAPRPTIQVIRPRPRPQRQAGQLAQLISAVNKLTMRAVPQQKPRRNRKNKKQRQKKQAPQNDPKQKKQPPQKKPAQKKKKPGRRERMCMKIENDCIFEVKHEGKVMGYACLVGDKVMKPAHVKGTIDNADLAKLAFKRSSKYDLECAQIPVHMKSDASKFTHEKPEGYYNWHHGAVQYSGGRFTIPTGAGKPGDSGRPIFDNKGRVVAIVLGGANEGARTALSVVTWNKDIVTKITPEGAEEWSLALPVLCLLANTTFPCSQPPCTPCCYEKEPESTLRMLEDNVMRPGYYQLLKASLTCSPHRQRRSTKDNFNVYKATRPYLAHCPDCGEGHSCHSPIALERIRNEATDGTLKIQVSLQIGIKTDDSHDWTKLRYMDSHTPADAERAGLLVRTSAPCTITGTMGHFILARCPKGETLTVGFTDSRKISHTCTHPFHHEPPVIGRERFHSRPQHGKELPCSTYVQSTAATAEEIEVHMPPDTPDRTLMTQQSGNVKITVNGQTVRYKCNCGGSNEGLTTTDKVINNCKIDQCHAAVTNHKNWQYNSPLVPRNAELGDRKGKIHIPFPLANVTCRVPKARNPTVTYGKNQVTMLLYPDHPTLLSYRNMGQEPNYHEEWVTHKKEVTLTVPTEGLEVTWGNNEPYKYWPQMSTNGTAHGHPHEIILYYYELYPTMTVVIVSVASFVLLSMVGTAVGMCVCARRRCITPYELTPGATVPFLLSLLCCVRTTKAATYYEAAAYLWNEQQPLFWLQALIPLAALIVLCNCLKLLPCCCKTLAFLAVMSIGAHTVSAYEHVTVIPNTVGVPYKTLVNRPGYSPMVLEMELQSVTLEPTLSLDYITCEYKTVIPSPYVKCCGTAECKDKSLPDYSCKVFTGVYPFMWGGAYCFCDAENTQLSEAHVEKSESCKTEFASAYRAHTASASAKLRVLYQGNNITVAAYANGDHAVTVKDAKFVVGPMSSAWTPFDNKIVVYKGDVYNMDYPPFGAGRPGQFGDIQSRTPESKDVYANTQLVLQRPAAGTVHVPYSQAPSGFKYWLKERGASLQHTAPFGCQIATNPVRAVNCAVGNIPISIDIPDAAFTRVVDAPSVTDMSCEVPACTHSSDFGGVAIIKYTASKKGKCAVHSMTNAVTIREADVEVEGNSQLQISFSTALASAEFRVQVCSTQVHCAAACHPPKDHIVNYPASHTTLGVQDISTTAMSWVQKITGGVGLIVAVAALILIVVLCVSFSRH

SEQ ID NO: 8 - protein, 1255 aa, Venezuelan equine encephalitis virus
MFPFQPMYPMQPMPYRNPFAAPRRPWFPRTDPFLAMQVQELTRSMANLTFKQRRDAPPEGPSAAKPKKEASQKQKGGGQGKKKKNQGKKKAKTGPPNPKAQNGNKKKTNKKPGKRQRMVMKLESDKTFPIMLEGKINGYACVVGGKLFRPMHVEGKIDNDVLAALKTKKASKYDLEYADVPQNMRADTFKYTHEKPQGYYSWHHGAVQYENGRFTVPKGVGAKGDSGRPILDNQGRVVAIVLGGVNEGSRTALSVVMWNEKGVTVKYTPENCEQWSLVTTMCLLANVTFPCAQPPICYDRKPAETLAMLSVNVDNPGYDELLEAAVKCPGRKRRSTEELFNEYKLTRPYMARCIRCAVGSCHSPIAIEAVKSDGHDGYVRLQTSSQYGLDSSGNLKGRTMRYDMHGTIKEIPLHQVSLYTSRPCHIVDGHGYFLLARCPAGDSITMEFKKDSVRHSCSVPYEVKFNPVGRELYTHPPEHGVEQACQVYAHDAQNRGAYVEMHLPGSEVDSSLVSLSGSSVTVTPPDGTSALVECECGGTKISETINKTKQFSQCTKKEQCRAYRLQNDKWVYNSDKLPKAAGATLKGKLHVPFLLADGKCTVPLAPEPMITFGFRSVSLKLHPKNPTYLITRQLADEPHYTHELISEPAVRNFTVTEKGWEFVWGNHPPKRFWAQETAPGNPHGLPHEVITHYYHRYPMSTILGLSICAAIATVSVAASTWLFCRSRVACLTPYRLTPNARIPFCLAVLCCARTARAETTWESLDHLWNNNQQMFWIQLLIPLAALIVVTRLLRCVCCVVPFLVMAGAAGAGAYEHATTMPSQAGISYNTIVNRAGYAPLPISITPTKIKLIPTVNLEYVTCHYKTGMDSPAIKCCGSQECTPTYRPDEQCKVFTGVYPFMWGGAYCFCDTENTQVSKAYVMKSDDCLADHAEAYKAHTASVQAFLNITVGEHSIVTTVYVNGETPVNFNGVKITAGPLSTAWTPFDRKIVQYAGEIYNYDFPEYGAGQPGAFGDIQSRTVSSSDLYANTNLVLQRPKAGAIHVPYTQAPSGFEQWKKDKAPSLKFTAPFGCEIYTNPIRAENCAVGSIPLAFDIPDALFTRVSETPTLSAAECTLNECVYSSDFGGIATVKYSASKSGKCAVHVPSGTATLKEAAVELTEQGSATIHFSTANIHPEFRLQICTSYVTCKGDCHPPKDHIVTHPQYHAQTFTAAVSKTAWTWLTSLLGGSAVIIIIGLVLATIVAMYVLTNQKHN

SEQ ID NO: 9 - protein, 61 aa, Chikungunya virus
ATYQEAAIYLWNEQQPLFWLQALIPLAALIVLCNCLRLLPCCCKTLAFLAVMSVGAHTVSA

SEQ ID NO: 10 - protein, 61 aa, Chikungunya virus
ATYYEAAAYLWNEQQPLFWLQALIPLAALIVLCNCLKLLPCCCKTLAFLAVMSIGAHTVSA

SEQ ID NO: 11 - protein, 56 aa, Venezuelan equine encephalitis virus
ETTWESLDHLWNNNQQMFWIQLLIPLAALIVVTRLLRCVCCVVPFLVMAGAAGAGA

SEQ ID NO: 12 - protein, 36 aa, synthetic construct
SGGADSFSLNDALAGSGNPNPQGYPGAWGNQPAGGS

SEQ ID NO: 13 - DNA, 96 bp, synthetic construct
  source 1..96: mol_type = other DNA
ggcgcggactctttttccttgaatgatgctctcgctgggtccggtaatcctaacccacaaggctatcctggagcgtggggcaatcaaccggcgggc

SEQ ID NO: 14 - protein, 16 aa, synthetic construct
KRPAATKKAGQAKKKK

SEQ ID NO: 15 - protein, 5 aa, synthetic construct
KKPKK

SEQ ID NO: 16 - protein, 8 aa, synthetic construct
RRNRKNKK